European Patent Application EP 4 273 245 A1, published November 8, 2023. Title: NUCLEIC ACID, PHARMACEUTICAL COMPOSITION AND SIRNA CONJUGATE CONTAINING THE NUCLEIC ACID, PREPARATION METHOD THEREFOR, AND USE THEREOF. Applicant: SUZHOU RIBO LIFE SCIENCE CO., LTD. The sequence listing filed with the application follows.

SEQUENCE LISTING (80 sequences)

SEQ ID NO: 1 - RNA, 19 nt, Artificial Sequence
  Sequence of nucleotide sequence I
cugaauuccaaaaaccaau

SEQ ID NO: 2 - RNA, 19 nt, Artificial Sequence
  Sequence of nucleotide sequence II
auugguuuuuggaauucag

SEQ ID NO: 3 - RNA, 19 nt, Artificial Sequence
  Sequence of nucleotide sequence I
  misc_feature (19)..(19): n is a, u, g or c
cugaauuccaaaaaccaan

SEQ ID NO: 4 - RNA, 19 nt, Artificial Sequence
  Sequence of nucleotide sequence II
  misc_feature (1)..(1): n is a, u, g or c
nuugguuuuuggaauucag

SEQ ID NO: 5 - RNA, 19 nt, Artificial Sequence
  Sequence of nucleotide sequence I
  misc_feature (19)..(19): n is a, u, g or c
cugaauuccaaaaaccaan

SEQ ID NO: 6 - RNA, 21 nt, Artificial Sequence
  Sequence of nucleotide sequence II
  misc_feature (1)..(1): n is a, u, g or c
nuugguuuuuggaauucagua

SEQ ID NO: 7 - RNA, 21 nt, Artificial Sequence
  Sequence of nucleotide sequence I
  misc_feature (21)..(21): n is a, u, g or c
uacugaauuccaaaaaccaan

SEQ ID NO: 8 - RNA, 23 nt, Artificial Sequence
  Sequence of nucleotide sequence II
  misc_feature (1)..(1): n is a, u, g or c
nuugguuuuuggaauucaguaua

SEQ ID NO: 9 - RNA, 19 nt, Artificial Sequence
  Sense strand of siPKKa1
cugaauuccaaaaaccaau

SEQ ID NO: 10 - RNA, 21 nt, Artificial Sequence
  Antisense strand of siPKKa1
auugguuuuuggaauucagua

SEQ ID NO: 11 - RNA, 21 nt, Artificial Sequence
  Sense strand of siPKKa2
uacugaauuccaaaaaccaau

SEQ ID NO: 12 - RNA, 23 nt, Artificial Sequence
  Antisense strand of siPKKa2
auugguuuuuggaauucaguaua

SEQ ID NO: 13 - RNA, 19 nt, Artificial Sequence
  Sense strand of siPKKa1-M1
cugaauuccaaaaaccaau

SEQ ID NO: 14 - RNA, 21 nt, Artificial Sequence
  Antisense strand of siPKKa1-M1
auugguuuuuggaauucagua

SEQ ID NO: 15 - RNA, 19 nt, Artificial Sequence
  Sense strand of siPKKa1-M2
cugaauuccaaaaaccaau

SEQ ID NO: 16 - RNA, 21 nt, Artificial Sequence
  Antisense strand of siPKKa1-M2
auugguuuuuggaauucagua

SEQ ID NO: 17 - RNA, 19 nt, Artificial Sequence
  Sense strand of siPKKa1-M3
cugaauuccaaaaaccaau

SEQ ID NO: 18 - RNA, 21 nt, Artificial Sequence
  Antisense strand of siPKKa1-M3
auugguuuuuggaauucagua

SEQ ID NO: 19 - RNA, 21 nt, Artificial Sequence
  Sense strand of siPKKa2-M1
uacugaauuccaaaaaccaau

SEQ ID NO: 20 - RNA, 23 nt, Artificial Sequence
  Antisense strand of siPKKa2-M1
auugguuuuuggaauucaguaua

SEQ ID NO: 21 - RNA, 21 nt, Artificial Sequence
  Sense strand of siPKKa2-M2
uacugaauuccaaaaaccaau

SEQ ID NO: 22 - RNA, 23 nt, Artificial Sequence
  Antisense strand of siPKKa2-M2
auugguuuuuggaauucaguaua

SEQ ID NO: 23 - RNA, 21 nt, Artificial Sequence
  Sense strand of siPKKa2-M3
uacugaauuccaaaaaccaau

SEQ ID NO: 24 - RNA, 23 nt, Artificial Sequence
  Antisense strand of siPKKa2-M3
auugguuuuuggaauucaguaua

SEQ ID NO: 25 - RNA, 19 nt, Artificial Sequence
  Sense strand of siPKKa1-M1S
cugaauuccaaaaaccaau

SEQ ID NO: 26 - RNA, 21 nt, Artificial Sequence
  Antisense strand of siPKKa1-M1S
auugguuuuuggaauucagua

SEQ ID NO: 27 - RNA, 19 nt, Artificial Sequence
  Sense strand of siPKKa1-M2S
cugaauuccaaaaaccaau

SEQ ID NO: 28 - RNA, 21 nt, Artificial Sequence
  Antisense strand of siPKKa1-M2S
auugguuuuuggaauucagua

SEQ ID NO: 29 - RNA, 19 nt, Artificial Sequence
  Sense strand of siPKKa1-M3S
cugaauuccaaaaaccaau

SEQ ID NO: 30 - RNA, 21 nt, Artificial Sequence
  Antisense strand of siPKKa1-M3S
auugguuuuuggaauucagua

SEQ ID NO: 31 - RNA, 21 nt, Artificial Sequence
  Sense strand of siPKKa2-M1S
uacugaauuccaaaaaccaau

SEQ ID NO: 32 - RNA, 23 nt, Artificial Sequence
  Antisense strand of siPKKa2-M1S
auugguuuuuggaauucaguaua

SEQ ID NO: 33 - RNA, 21 nt, Artificial Sequence
  Sense strand of siPKKa2-M2S
uacugaauuccaaaaaccaau

SEQ ID NO: 34 - RNA, 23 nt, Artificial Sequence
  Antisense strand of siPKKa2-M2S
auugguuuuuggaauucaguaua

SEQ ID NO: 35 - RNA, 21 nt, Artificial Sequence
  Sense strand of siPKKa2-M3S
uacugaauuccaaaaaccaau

SEQ ID NO: 36 - RNA, 23 nt, Artificial Sequence
  Antisense strand of siPKKa2-M3S
auugguuuuuggaauucaguaua

SEQ ID NO: 37 - RNA, 19 nt, Artificial Sequence
  Sense strand of siPKKa1-M1P1
cugaauuccaaaaaccaau

SEQ ID NO: 38 - RNA, 21 nt, Artificial Sequence
  Antisense strand of siPKKa1-M1P1
auugguuuuuggaauucagua

SEQ ID NO: 39 - RNA, 19 nt, Artificial Sequence
  Sense strand of siPKKa1-M2P1
cugaauuccaaaaaccaau

SEQ ID NO: 40 - RNA, 21 nt, Artificial Sequence
  Antisense strand of siPKKa1-M2P1
auugguuuuuggaauucagua

SEQ ID NO: 41 - RNA, 19 nt, Artificial Sequence
  Sense strand of siPKKa1-M3P1
cugaauuccaaaaaccaau

SEQ ID NO: 42 - RNA, 21 nt, Artificial Sequence
  Antisense strand of siPKKa1-M3P1
auugguuuuuggaauucagua

SEQ ID NO: 43 - RNA, 21 nt, Artificial Sequence
  Sense strand of siPKKa2-M1P1
uacugaauuccaaaaaccaau

SEQ ID NO: 44 - RNA, 23 nt, Artificial Sequence
  Antisense strand of siPKKa2-M1P1
auugguuuuuggaauucaguaua

SEQ ID NO: 45 - RNA, 21 nt, Artificial Sequence
  Sense strand of siPKKa2-M2P1
uacugaauuccaaaaaccaau

SEQ ID NO: 46 - RNA, 23 nt, Artificial Sequence
  Antisense strand of siPKKa2-M2P1
auugguuuuuggaauucaguaua

SEQ ID NO: 47 - RNA, 21 nt, Artificial Sequence
  Sense strand of siPKKa2-M3P1
uacugaauuccaaaaaccaau

SEQ ID NO: 48 - RNA, 23 nt, Artificial Sequence
  Antisense strand of siPKKa2-M3P1
auugguuuuuggaauucaguaua

SEQ ID NO: 49 - RNA, 19 nt, Artificial Sequence
  Sense strand of siPKKa1-M1SP1
cugaauuccaaaaaccaau

SEQ ID NO: 50 - RNA, 21 nt, Artificial Sequence
  Antisense strand of siPKKa1-M1SP1
auugguuuuuggaauucagua

SEQ ID NO: 51 - RNA, 19 nt, Artificial Sequence
  Sense strand of siPKKa1-M2SP1
cugaauuccaaaaaccaau

SEQ ID NO: 52 - RNA, 21 nt, Artificial Sequence
  Antisense strand of siPKKa1-M2SP1
auugguuuuuggaauucagua

SEQ ID NO: 53 - RNA, 19 nt, Artificial Sequence
  Sense strand of siPKKa1-M3SP1
cugaauuccaaaaaccaau

SEQ ID NO: 54 - RNA, 21 nt, Artificial Sequence
  Antisense strand of siPKKa1-M3SP1
auugguuuuuggaauucagua

SEQ ID NO: 55 - RNA, 21 nt, Artificial Sequence
  Sense strand of siPKKa2-M1SP1
uacugaauuccaaaaaccaau

SEQ ID NO: 56 - RNA, 23 nt, Artificial Sequence
  Antisense strand of siPKKa2-M1SP1
auugguuuuuggaauucaguaua

SEQ ID NO: 57 - RNA, 21 nt, Artificial Sequence
  Sense strand of siPKKa2-M2SP1
uacugaauuccaaaaaccaau

SEQ ID NO: 58 - RNA, 23 nt, Artificial Sequence
  Antisense strand of siPKKa2-M2SP1
auugguuuuuggaauucaguaua

SEQ ID NO: 59 - RNA, 21 nt, Artificial Sequence
  Sense strand of siPKKa2-M3SP1
uacugaauuccaaaaaccaau

SEQ ID NO: 60 - RNA, 23 nt, Artificial Sequence
  Antisense strand of siPKKa2-M3SP1
auugguuuuuggaauucaguaua

SEQ ID NO: 61 - RNA, 19 nt, Artificial Sequence
  Sense strand of siPKKa1M1S
cugaauuccaaaaaccaau

SEQ ID NO: 62 - RNA, 21 nt, Artificial Sequence
  Antisense strand of siPKKa1M1S
auugguuuuuggaauucagua

SEQ ID NO: 63 - RNA, 19 nt, Artificial Sequence
  Sense strand of siPKKa1M1S
cugaauuccaaaaaccaau

SEQ ID NO: 64 - RNA, 21 nt, Artificial Sequence
  Antisense strand of siPKKa1M1S
auugguuuuuggaauucagua

SEQ ID NO: 65 - RNA, 19 nt, Artificial Sequence
  Sense strand of NC
uucuccgaacgugucacgu

SEQ ID NO: 66 - RNA, 19 nt, Artificial Sequence
  Antisense strand of NC
acgugacacguucggagaa

SEQ ID NO: 67 - DNA, 20 bp, Artificial Sequence
  Upstream primer of PKK in mice
tgccttccaaagctgacaca

SEQ ID NO: 68 - DNA, 20 bp, Artificial Sequence
  Downstream primer of PKK in mice
gtgatacccaccaactgcca

SEQ ID NO: 69 - DNA, 24 bp, Artificial Sequence
  Upstream primer of GAPDH in mice
aactttggcattgtggaagggctc

SEQ ID NO: 70 - DNA, 24 bp, Artificial Sequence
  Downstream primer of GAPDH in mice
tggaagagtgggagttgctgttga

SEQ ID NO: 71 - DNA, 19 bp, Artificial Sequence
  Upstream primer of GAPDH in mice
tgcaccaccaactgcttag

SEQ ID NO: 72 - DNA, 19 bp, Artificial Sequence
  Downstream primer of GAPDH in mice
ggatgcagggatgatgttc

SEQ ID NO: 73 - DNA, 20 bp, Artificial Sequence
  Upstream primer of PKK in mice
tgccttccaaagctgacaca

SEQ ID NO: 74 - DNA, 20 bp, Artificial Sequence
  Downstream primer of PKK in mice
gtgatacccaccaactgcca

SEQ ID NO: 75 - RNA, 21 nt, Artificial Sequence
  Sense strand of siPKKa2M4
uacugaauuccaaaaaccaau

SEQ ID NO: 76 - RNA, 23 nt, Artificial Sequence
  Antiense strand of siPKKa2M4
auugguuuuuggaauucaguaua

SEQ ID NO: 77 - RNA, 19 nt, Artificial Sequence
  Sense strand of siPKKa
cugaauuccaaaaaccaau

SEQ ID NO: 78 - RNA, 19 nt, Artificial Sequence
  Antisense strand of siPKKa
auugguuuuuggaauucag

SEQ ID NO: 79 - RNA, 21 nt, Artificial Sequence
  Sense strand of siPKKa3
uacugaauuccaaaaaccaaa

SEQ ID NO: 80 - RNA, 23 nt, Artificial Sequence
  Antisense strand of siPKKa3
uuugguuuuuggaauucaguaua